European Patent Application EP 4 722 244 A1, published April 8, 2026. Title: Anti-TLR2 Antibody and Use Thereof. Applicant: Neuramedy Co., LTD. The sequence listing filed with the application follows.

SEQUENCE LISTING (10 sequences)

SEQ ID NO: 1 - protein, 6 aa, synthetic construct
  source 1..6: note = NM-103 heavy chain CDR1
TTYGIN

SEQ ID NO: 2 - protein, 18 aa, synthetic construct
  source 1..18: note = NM-103 heavy chain CDR2
GWIYPRDGSTNFNENFKD

SEQ ID NO: 3 - protein, 9 aa, synthetic construct
  source 1..9: note = NM-103 heavy chain CDR3
LTGGTFLDY

SEQ ID NO: 4 - protein, 15 aa, synthetic construct
  source 1..15: note = NM-103 light chain CDR1
RASESVEYYGTSLMQ

SEQ ID NO: 5 - protein, 7 aa, synthetic construct
  source 1..7: note = NM-103 light chain CDR2
GASNVES

SEQ ID NO: 6 - protein, 9 aa, synthetic construct
  source 1..9: note = NM-103 light chain CDR3
QQSRKLPWT

SEQ ID NO: 7 - protein, 118 aa, synthetic construct
  source 1..118: note = NM-103 heavy chain variable region
QVQLVQSGSELKKPGASVKLSCKASGFTFTTYGINWVRQAPGQGLEWIGWIYPRDGSTNFNENFKDRATITVDTSASTAYMELSSLRSEDTAVYFCARLTGGTFLDYWGQGTTVTVSS

SEQ ID NO: 8 - protein, 111 aa, synthetic construct
  source 1..111: note = NM-103 light chain variable region
DIVLTQSPATLSLSPGERATLSCRASESVEYYGTSLMQWYQQKPGQPPKLLIFGASNVESGVPDRFSGSGSGTDFTLKISRVEAEDVGMYFCQQSRKLPWTFGGGTKVEIK

SEQ ID NO: 9 - protein, 445 aa, synthetic construct
  source 1..445: note = NM-103 heavy chain
QVQLVQSGSELKKPGASVKLSCKASGFTFTTYGINWVRQAPGQGLEWIGWIYPRDGSTNFNENFKDRATITVDTSASTAYMELSSLRSEDTAVYFCARLTGGTFLDYWGQGTTVTVSSASTKGPSVFPLAPCSRSTSESTAALGCLVKDYFPEPVTVSWNSGALTSGVHTFPAVLQSSGLYSLSSVVTVPSSSLGTKTYTCNVDHKPSNTKVDKRVESKYGPPCPPCPAPEFLGGPSVFLFPPKPKDTLMISRTPEVTCVVVDVSQEDPEVQFNWYVDGVEVHNAKTKPREEQFNSTYRVVSVLTVLHQDWLNGKEYKCKVSNKGLPSSIEKTISKAKGQPREPQVYTLPPSQEEMTKNQVSLTCLVKGFYPSDIAVEWESNGQPENNYKTTPPVLDSDGSFFLYSRLTVDKSRWQEGNVFSCSVMHEALHNHYTQKSLSLSLGK

SEQ ID NO: 10 - protein, 218 aa, synthetic construct
  source 1..218: note = NM-103 light chain
DIVLTQSPATLSLSPGERATLSCRASESVEYYGTSLMQWYQQKPGQPPKLLIFGASNVESGVPDRFSGSGSGTDFTLKISRVEAEDVGMYFCQQSRKLPWTFGGGTKVEIKRTVAAPSVFIFPPSDEQLKSGTASVVCLLNNFYPREAKVQWKVDNALQSGNSQESVTEQDSKDSTYSLSSTLTLSKADYEKHKVYACEVTHQGLSSPVTKSFNRGEC